European Patent Application EP 4 454 640 A2, published October 30, 2024. Title: IMPROVED LIPID NANOPARTICLES FOR DELIVERY OF NUCLEIC ACIDS. Applicant: Acuitas Therapeutics, Inc. Application EP, filed August 14, 2020. The sequence listing filed with the application follows.

SEQUENCE LISTING (1 sequence)

SEQ ID NO: 1 - DNA, 16 bp, synthetic construct
  source 1..16: mol_type = other DNA
taacgttgaggggcat